European Patent Specification EP 3 416 681 B1, published January 21, 2026. Title: NOVEL ANTIGEN FOR USE IN MALARIA VACCINE. Applicant: CAMRIS INTERNATIONAL, INC. The sequence listing filed with the application follows.

SEQUENCE LISTING (9 sequences)

SEQ ID NO: 1 - protein, 816 aa, Plasmodium yoelii
MGDVDNVLISIKKIESIKSQLNQLNKIIQNEFGSYCGRKNRSINLEIHHNEFDKSIFKRLYSSWRMEDLNNFNGKSVIKIMERNPYVIFFFFFIMIFIIVYLISFILYTKWFKKLLKKFSNSHKNNKDKEEDWVKKNKAYRNSNSTHGTINKDNYNQELDELHNSDENEENSNVINIVKKRAYNLVINLIVCSFLICLIFLGIWTIFIFADTQKGINMNICGLSKTVEQFLIDKCPDTKNVNPQCYSLEHVINDAVSVMNQYQLTKEFVKNKTNLNKNKGLPIVLKYQTGFNMLAKLRDNIDKNVKKLENGYLHTYPVLTKLRFTLDEIVSKGENLLNQAESIIDSSKEEIGKIFNNVDNAIANTVHNNVPSLSSKISGLGIYIKKQDENLKIRYILNKFTVTMIILSIVILLFSLLVLIGMLSYMYFLIRGHSINEKFFSKLLGFFSGTFGFLAIIILIIGTALLSLSVLGGTSCIISDRILKNEFTFDFLSENKIGYCLQNPDESIINKNIVKKYANTLDSLNTNDIYNSVEGYSGYFDKIKDEYKQHSKIINENMWIIIPTDNNKYVKNVKSDIIKKSLLGTCLTKESAQFEEYHLMGTDAYMKYINKFGLLNNYEMCFEDPSCENNDRKYNINYNSKVTDPKYLDVKRNRVMLYQDSDFDNVLEVFILKSKINNDKIFNISDLDETKKENITWREYTPKNGAGENKKSIVQTYFEKAIEYMKFENVLTLLKEVNNHINSFKNVIIEKANSLVDNTNCSRFINVLTNIRHNYCDNGILKLTRLSVILISCGFVSFCLWYLFLFFWIYHQMKII

SEQ ID NO: 2 - DNA, 2451 bp, Plasmodium yoelii
atgggagacgttgacaatgtgttaataagtatcaaaaaaatagaatcaataaaaagccaattaaaccagttaaacaaaattatacaaaatgaatttgggtcttattgtgggcgaaaaaatagaagtataaatcttgaaatacatcataatgaatttgataaaagtatattcaaacgtttatattcatcatggagaatggaagatcttaataattttaacgggaaaagtgttataaaaataatggaaagaaatccatatgttatatttttttttttttttataatgatttttattattgtttatttaatttcatttattttgtatactaaatggtttaaaaaattattaaaaaaattttcgaattcacacaaaaataataaagataaagaagaagattgggtaaaaaaaaataaagcttatagaaattctaatagcacacatggtactattaataaggataattataatcaggaacttgatgagcttcataatagtgatgaaaatgaagaaaatagtaatgttataaatattgtaaaaaagagagcttataatttagtaattaatttgatagtttgttcttttcttatttgtcttatttttttgggaatttggacaatatttatttttgcagatacacaaaaaggaattaatatgaatatctgtggattatcaaaaacagttgaacagtttcttattgataaatgccccgacacaaaaaatgtaaatccacaatgttattctttagagcatgttattaatgatgctgtttcagtaatgaatcagtatcaactcaccaaagaatttgttaaaaataaaacgaatttgaacaagaataagggcttgcctattgttttaaagtaccaaaccggattcaacatgctagcaaaacttagagacaacatagataaaaatgttaaaaaattagagaacggatatcttcacacatatccagttttaacaaaacttagatttactttggatgaaattgtttcgaagggagagaatctattaaatcaggctgaatctattattgattcttcaaaagaagaaattggaaaaatattcaataatgtagataatgctatagctaatactgtacataataatgttccgtctttatcatcaaaaataagtggattaggaatatatataaaaaaacaagacgaaaatttaaaaatacgatatatattaaataaatttacagttacaatgataattttaagtatagtcatattattattttcattacttgtgttaataggaatgttatcttatatgtattttttaataagaggccattcaataaatgaaaaatttttttcaaaattacttggtttttttagtggaacatttggatttttagcaattataattttaataataggtacggcattattaagtttatctgttttgggtggaacaagttgtattatatctgatcgaatattaaaaaatgaatttacttttgattttttaagcgaaaataaaattggttattgtttacagaatccagatgaatctattattaataaaaatattgtaaaaaaatatgcaaacactcttgactctttaaatacaaatgatatatataatagtgttgaaggctatagtggttattttgataaaattaaggatgaatataaacaacattctaaaattataaatgaaaatatgtggataattattcctacagataataataaatatgtaaaaaatgttaaatcagatattattaaaaaatcattattaggaacatgtttaacaaaagaaagtgcccaatttgaagagtatcatcttatgggaacagatgcttatatgaaatatataaataaatttggtttgctaaataattatgagatgtgttttgaagacccatcatgtgaaaataacgacagaaaatacaatatcaattataactctaaagttacagacccaaaatatcttgatgttaaacgtaatagagtcatgctttatcaagatagcgattttgataatgtacttgaagtgttcatattaaaatcaaaaattaataatgataaaatttttaatattagcgatttagatgaaacaaagaaggaaaatataacatggagagaatatacaccaaaaaatggagccggagaaaataaaaaatctattgttcaaacatattttgagaaagctattgaatatatgaaatttgaaaatgttttaactttacttaaagaagttaataatcatataaattcatttaaaaatgttattattgaaaaagctaattcattagtagataatacaaattgtagtagatttattaatgtactaactaatataagacataattattgtgacaatggaattttaaaattaactcgattatcagtcatacttatttcatgtggatttgtttccttttgtctttggtaccttttcctttttttttggatataccatcaaatgaagattatttga

SEQ ID NO: 3 - protein, 791 aa, Plasmodium falciparum
MVDFNDLSVELKKTELIKEDLRNLSHIINNEFSYFCQNENKNVSFNNNISSYYNDDIFSKSTLNNLYTSWKLEDFSHFDFSSILDILKRNQYVMCSIYFLLIFSCIYFLTLLLYTKCIKTTLKKWFCRYCSENINENNSNHNEQRTVLQNVINKSCYFITYSSIICLLLFLLLSGITYMHYFIKTKKGIHSNICNIYTRLDKFLLNKCLDPKKVDTSCYSAEHILNDLSSILEEYKKVKQQAKDDTLLDENTPFPLLERYITTFNKLNVLKNNINKNNTTLENEYFHTYPALKGISETLTTIISEGNKNFGNARNVIKEVKSTIKYSFHTVDETIRNVFKDSVPKITGLITQAGKSIKGINNKYKIKERIPKYTNIILLTNIILLLPPFLILLGIIIFMIFILMGYIQKNNNFFIKLFGHFSAYFGLLTIIILSFGILFLSTSVIGGTSCILSERILKNELRFDILNNTLIDYCIKNESAPLIDDDITTSFVAKINSFDTGHIDHNINEYEKHFTILKESFFHKSLKFMDYIWIVIMKRENNTFLNRIRTEQVKKSLLITGIINENIKYENMEAIGIRSYLTTLNKIIFPENNGKICFNDIICEKENNTYNITENSKTTDQKYRNIRDGMDEHLRNDLDAIVQLFVYKARILKENIFDINDLDSNEKNKIGWSEYTPRNINGTQKKSIINTFLVNVIESINFSEIINFFDKMRDQFNVLKDLILLKIDTLTENTKCNKLVKELINVRKDYCNNVVLNLSTLSVYLIIFSITSFLLWYLFLFLWFYYNIKPS

SEQ ID NO: 4 - DNA, 2375 bp, Plasmodium falciparum
atggtagacttcaacgatttaagcgttgaactaaaaaaaacagaattaataaaagaggacctgagaaatctaagccatataataaataatgaatttagttacttttgtcaaaatgaaaacaagaacgtatctttcaacaataatattagtagttattataatgatgatatattttctaaaagtacattaaataatttatatacatcttggaaattagaagatttttctcattttgatttcagtagtattttagatatattaaaaagaaatcaatatgttatgtgtagtatatatttcctcctaattttttcttgtatctattttttaacattattattatatacaaaatgtataaaaacaacgttaaaaaaatggttctgtagatattgtagtgaaaatataaatgaaaataatagtaatcataatgaacaaagaacagtattacaaaatgttataaataaatcatgttattttattacttattcatctataatctgtcttttattatttcttctactttctggaattacatatatgcattattttataaaaacaaaaaaaggaatacattctaatatttgtaatatttatacaaggcttgataaattcttattaaataaatgtctagatccaaaaaaagttgatacctcgtgttattcagctgaacatatattgaatgatctttcttccatattggaagaatataaaaaggtgaagcaacaagcaaaggacgacacgttgcttgacgagaacactcccttccccctactcgaaagatacattacaacgttcaataagctaaatgtactaaaaaacaatataaataaaaataacacaacactcgaaaacgaatacttccacacatatccagccctcaaaggaatcagcgaaacactaacaaccattattagtgaaggcaataaaaatttcggaaatgccagaaatgttattaaagaagttaaaagcacaataaaatattcgtttcatactgttgacgaaaccataagaaatgtatttaaagatagtgtacctaaaattacaggattaataacacaagctgggaaatctatcaaaggaataaataacaaatataaaattaaagagcgtattcctaaatatacaaatattattttattaactaatattattttattgttaccaccattcttaatattattaggtatcataatttttatgatatttattcttatgggatatatacaaaaaaataataatttcttcataaaattatttggtcatttcagtgcttactttggtttactcactataattattttatcctttggaatactattcttaagtacttcagtcataggaggcacatcttgtattttatcagaaagaattttaaaaaatgaattacgttttgatatattaaataatactcttatagattattgtattaaaaatgaaagcgcaccattaattgacgatgatataacaacaagctttgtcgctaaaattaattctttcgatacaggacatatagatcataatataaacgaatatgaaaaacattttacaattttaaaagaatctttttttcataagtcattaaaatttatggattatatatggattgttataatgaaacgagaaaataatacatttttaaatagaataagaactgaacaagtcaaaaaatcgttattaataacaggtattataaacgaaaatattaaatatgaaaatatggaagctataggtatcagatcctatttaactacgttgaacaaaattatttttcctgaaaataatggtaaaatatgttttaatgatatcatatgtgaaaaggagaataatacatataatattactgagaattcaaaaacaaccgatcagaaatatagaaatatacgtgatggaatggatgaacatcttagaaacgatttggatgctttgttcaactctttgtttataaagcacgtattctaaaagaaaatatattcgatattaacgatcttgatagtaacgaaaaaaacaaaataggatggagcgaatatacacccagaaatataaatggaacacaaaaaaaatcaatcattaatactttcctagtaaatgttattgaaagtattaacttttcagaaataataaatttctttgataaaatgagagatcaatttaatgtacttaaagacctaattctattaaaaattgatacattaacagaaaatacaaaatgtaataaattagtaaaagaacttattaatgtcagaaaagattattgtaataacgtcgttttgaatttatctactttatctgtatatttaattatattttccatcacttcatttttattatggtatctatttctattcttgtggttctattataatattaaaccatcatag

SEQ ID NO: 5 - DNA, 2370 bp, Plasmodium vivax
atgagcgacgagtacaacctgagcatcgacctgaagaagacggagctgctgaaggagcacttgaaagccattgccaaagttatgcacaatgagttcgggtacttttgccccagtggtggagtgaaggtcccgcaggaccaccccaatgaattctcgaagaccatatggagcatcctttacacgtcctggaggatggaagattttacgaggctgaatttaaaaagcgttttgaacatcctcaagaggaacccctacgtgatggggtgtgtgtacttcctcatcatcttcacgtgtgtatatctgttaacgttattcctgtataccaagtgctttcggaggttgattaaagccattcgttgcaaaacgtgtaggaggaagaaacagaagcgagaacaacaggagagtgaaaataaagatttaattgaaaatgtgaagaagcgattctttaacatcatgacgtacgtgtttttgagttcgcttctgtgtgttctgattggtttgggcatctggtatatgatttcttttttcaaaacgaggaatgggatttatatgaatgtatgcagcgcgtccacctcgattgagaacttcctcaccgaccgctgctccgtgcagggcggcgaggtggactcgtcgtgctactccctggagcacatcgtgagcgacgcggtgtccatcgtggagcagtaccaagacatcaagctgcagataaaggcggacctgctggtggacgaggacagggcggttccgctcctcacaggcttcctcaccgtgttcgagaacctgaagaagctgcagcagaacgtggcgcggaacaaccacatcctggaggagcagtacttccacacgtaccccgtgctgacgaggctgggcagagcgctcgacgcagtcatccaggagggagaggcgaacctccagcaggcgacaggcaccctcgatgaagccaagcaagcagtcaaaggagccttcgaagaaatcgaccaagttctgggagcaacctttaaagaaaatatggaaaaggtaaatgacaaaattacgctcttcaataagtctataaatagaataatacaccagtataagataaagcaaaatttgaagaagtacacgatttcaattttgattgtgaagttggttttgctcattcctccccttctcattctaattgggttagtgcttttcatattctttttggtgaaaggggacattggaaacagcagtcatttttttttggacctctttggagtgttcagcgcctactttggatttttgacgatcgtcattttgctaatcgggatagcaatgctgagtgcgtccatcttgggggggacgacctgcatcatcgccgatagggttttaaaaaatgagctgaactttgacgtgctgaatgataccctgatcgattactgcctgaagaatgaggagtcgccccttctctcggaggacatcaccaaggggcttgtagacaacatgaagtctttggacaccaccgaaatggagaggagggtgaatgaatacgattcctatttcaacgatatgaagagaaccttccgcgaaaatacaagaaattttgtcaactacatgtgggtggtcattaccaagccgaacaacaacctgtatgtggatcgaattcggctaaacactctgaaaaagtccctcctagcgaccagcatcactcgggacaatatcaaatttggtaaattcaacctctggggaacagatgaatactttgaaaatctgaatcgccactattttaggggcacccagtttgccctctgctttgaaaatgaagaatgcgacagggaggaggacaagtttaacatcaactttaggtcctccataaatgaccccaagtaccagaggatgaggaaccacctcaggaataatgatcttagagaggacctagacaacgtggtggagctattcatttacaagtctagagttaggaccgaaaagatattctctgtggacgacttggatagcagcatgacggacaaaatagggtggagtgagtacacgccgaggattaacaaaagggagggggggaaagaacaaaccttcattttgaggaagtacctcgtggaggacattgaaaatttgaacttcaaagacgtggttagcttcttcgagaaaattaaacagaaattcaacaccctcagagacacgatcattacgaaggtgcagatgctcgtgaagaacaccaactgcagcagactcgttggcgagatgcacaatttgaaacacatctactgcgaccgagtcgtgctgaacatgaccatcctctccgtcgcgctcgtctccttctccatcatttcgttcttcctctggtactgctttttgttcttttggctgtactaccagatgaagatgatgtga

SEQ ID NO: 6 - protein, 789 aa, Plasmodium vivax
MSDEYNLSIDLKKTELLKEHLKAIAKVMHNEFGYFCPSGGVKVPQDHPNEFSKTIWSILYTSWRMEDFTRLNLKSVLNILKRNPYVMGCVYFLIIFTCVYLLTLFLYTKCFRRLIKAIRCKTCRRKKQKREQQESENKDLIENVKKRFFNIMTYVFLSSLLCVLIGLGIWYMISFFKTRNGIYMNVCSASTSIENFLTDRCSVQGGEVDSSCYSLEHIVSDAVSIVEQYQDIKLQIKADLLVDEDRAVPLLTGFLTVFENLKKLQQNVARNNHILEEQYFHTYPVLTRLGRALDAVIQEGEANLQQATGTLDEAKQAVKGAFEEIDQVLGATFKENMEKVNDKITLFNKSINRIIHQYKIKQNLKKYTISILIVKLVLLIPPLLILIGLVLFIFFLVKGDIGNSSHFFLDLFGVFSAYFGFLTIVILLIGIAMLSASILGGTTCIIADRVLKNELNFDVLNDTLIDYCLKNEESPLLSEDITKGLVDNMKSLDTTEMERRVNEYDSYFNDMKRTFRENTRNFVNYMWVVITKPNNNLYVDRIRLNTLKKSLLATSITRDNIKFGKFNLWGTDEYFENLNRHYFRGTQFALCFENEECDREEDKFNINFRSSINDPKYQRMRNHLRNNDLREDLDNVVELFIYKSRVRTEKIFSVDDLDSSMTDKIGWSEYTPRINKREGGKEQTFILRKYLVEDIENLNFKDVVSFFEKIKQKFNTLRDTIITKVQMLVKNTNCSRLVGEMHNLKHIYCDRVVLNMTILSVALVSFSIISFFLWYCFLFFWLYYQMKMM

SEQ ID NO: 7 - protein, 413 aa, Plasmodium falciparum
MNLLVFFCFFLLSCIVHLSRCSDNNSYSFEIVNRSTWLNIAERIFKGNAPFNFTIIPYNYVNNSTEENNNKDSVLLISKNLKNSSNPVDENNHIIDSTKKNTSNNNNNNSNIVGIYESQVHEEKIKEDNTRQDNINKKENEIINNNHQIPVSNIFSENIDNNKNYIESNYKSTYNNNPELIHSTDFIGSNNNHTFNFLSRYNNSVLNNMQGNTKVPGNVPELKARIFSEEENTEVESAENNHTNSLNPNESCDQIIKLGDIINSVNEKIISINSTVNNVLCINLDSVNGNGFVWTLLGVHKKKPLIDPSNFPTKRVTQSYVSPDISVTNPVPIPKNSNTNKDDSINNKQDGSQNNTTTNHFPKPREQLVGGSSMLISKIKPHKPGKYFIVYSYYRPFDPTRDTNTRIVELNVQ

SEQ ID NO: 8 - protein, 397 aa, Plasmodium falciparum
MMRKLAILSVSSFLFVEALFQEYQCYGSSSNTRVLNELNYDNAGTNLYNELEMNYYGKQENWYSLKKNSRSLGENDDGNNEDNEKLRKPKHKKLKQPADGNPDPNANPNVDPNANPNVDPNANPNVDPNANPNANPNANPNANPNANPNANPNANPNANPNANPNANPNANPNANPNANPNANPNANPNANPNANPNVDPNANPNANPNANPNANPNANPNANPNANPNANPNANPNANPNANPNANPNANPNANPNANPNANPNANPNANPNKNNQGNGQGHNMPNDPNRNVDENANANSAVKNNNNEEPSDKHIKEYLNKIQNSLSTEWSPCSVTCGNGIQVRIKPGSANKPKDELDYANDIEKKICKMEKCSSVFNVVNSSIGLIMVLSFLFLN

SEQ ID NO: 9 - protein, 229 aa, Plasmodium falciparum
MKVSKLVLFAHIFFIINILCQYICLNASKVNKKGKIAEEKKRKNIKNIDKAIEEHNKRKKLIYYSLIASGAIASVAAILGLGYYGYKKSREDDLYYNKYLEYRNGEYNIKYQDGAIASTSEFYIEPEGINKINLNKPIIENKNNVDVSIKRYNNFVDIARLSIQKHFEHLSNDQKDSHVNNMEYMQKFVQGLQENRNISLSKYQENKAVMDLKYHLQKVYANYLSQEEN